European Patent Application EP 4 197 550 A1, published June 21, 2023. Title: A composition comprising a trigonal glucagon/GLP-1/GIP receptor agonist for lowering blood pressure. Applicant: HANMI PHARM. CO., LTD. The sequence listing filed with the application follows.

SEQUENCE LISTING (124 sequences)

SEQ ID NO: 1 - protein, 30 aa, Artificial Sequence
  Trigonal agonist
  MISC_FEATURE (2): Xaa is aminoisobutyric acid (Aib)
HXQGTFTSDVSSYLDGQAAKEFIAWLVKGC

SEQ ID NO: 2 - protein, 30 aa, Artificial Sequence
  Trigonal agonist
  MISC_FEATURE (2): Xaa is aminoisobutyric acid (Aib)
HXQGTFTSDVSSYLDGQAQKEFIAWLVKGC

SEQ ID NO: 3 - protein, 41 aa, Artificial Sequence
  Trigonal agonist
  MISC_FEATURE (2): Xaa is aminoisobutyric acid (Aib)
HXQGTFTSDVSSYLLGQAAKQFIAWLVKGGGPSSGAPPPSC

SEQ ID NO: 4 - protein, 30 aa, Artificial Sequence
  Trigonal agonist
  MISC_FEATURE (2): Xaa is aminoisobutyric acid (Aib)
HXQGTFTSDVSSYLLGQQQKEFIAWLVKGC

SEQ ID NO: 5 - protein, 41 aa, Artificial Sequence
  Trigonal agonist
  MISC_FEATURE (2): Xaa is aminoisobutyric acid (Aib)
HXQGTFTSDVSSYLLGQQQKEFIAWLVKGGGPSSGAPPPSC

SEQ ID NO: 6 - protein, 30 aa, Artificial Sequence
  Trigonal agonist
  MISC_FEATURE (2): Xaa is aminoisobutyric acid (Aib)
HXQGTFTSDVSSYLDGQAAKEFVAWLLKGC

SEQ ID NO: 7 - protein, 30 aa, Artificial Sequence
  Trigonal agonist
  MISC_FEATURE (2): Xaa is aminoisobutyric acid (Aib)
HXQGTFTSDVSKYLDGQAAKEFVAWLLKGC

SEQ ID NO: 8 - protein, 30 aa, Artificial Sequence
  Trigonal agonist
  MISC_FEATURE (2): Xaa is aminoisobutyric acid (Aib)
HXQGTFTSDVSKYLDGQAAQEFVAWLLKGC

SEQ ID NO: 9 - protein, 30 aa, Artificial Sequence
  Trigonal agonist
  MISC_FEATURE (2): Xaa is aminoisobutyric acid (Aib)
HXQGTFTSDVSKYLDGQAAQEFVAWLLAGC

SEQ ID NO: 10 - protein, 41 aa, Artificial Sequence
  Trigonal agonist
  MISC_FEATURE (2): Xaa is aminoisobutyric acid (Aib)
HXQGTFTSDVSKYLDGQAAQEFVAWLLAGGGPSSGAPPPSC

SEQ ID NO: 11 - protein, 41 aa, Artificial Sequence
  Trigonal agonist
  MISC_FEATURE (1): Xaa is 4-imidazoacetyl (CA)
XGEGTFTSDLSKYLDSRRQQLFVQWLKAGGPSSGAPPPSHG

SEQ ID NO: 12 - protein, 41 aa, Artificial Sequence
  Trigonal agonist
  MISC_FEATURE (1): Xaa is 4-imidazoacetyl (CA)
XGEGTFISDLSKYMDEQAVQLFVEWLMAGGPSSGAPPPSHG

SEQ ID NO: 13 - protein, 41 aa, Artificial Sequence
  Trigonal agonist
  MISC_FEATURE (1): Xaa is 4-imidazoacetyl (CA)
XGEGTFISDYSIQLDEIAVQDFVEWLLAQKPSSGAPPPSHG

SEQ ID NO: 14 - protein, 41 aa, Artificial Sequence
  Trigonal agonist
  MISC_FEATURE (1): Xaa is 4-imidazoacetyl (CA)
XGQGTFTSDYSIQLDEIAVRDFVEWLKNGGPSSGAPPPSHG

SEQ ID NO: 15 - protein, 41 aa, Artificial Sequence
  Trigonal agonist
  MISC_FEATURE (1): Xaa is 4-imidazoacetyl (CA)
XGQGTFTSDLSKQMDEEAVRLFIEWLKNGGPSSGAPPPSHG

SEQ ID NO: 16 - protein, 41 aa, Artificial Sequence
  Trigonal agonist
  MISC_FEATURE (1): Xaa is 4-imidazoacetyl (CA)
XGQGTFTSDLSKQMDSEAQQLFIEWLKNGGPSSGAPPPSHG

SEQ ID NO: 17 - protein, 41 aa, Artificial Sequence
  Trigonal agonist
  MISC_FEATURE (1): Xaa is 4-imidazoacetyl (CA)
XGQGTFTSDLSKQMDEERAREFIEWLLAQKPSSGAPPPSHG

SEQ ID NO: 18 - protein, 41 aa, Artificial Sequence
  Trigonal agonist
  MISC_FEATURE (1): Xaa is 4-imidazoacetyl (CA)
XGQGTFTSDLSKQMDSERAREFIEWLKNTGPSSGAPPPSHG

SEQ ID NO: 19 - protein, 41 aa, Artificial Sequence
  Trigonal agonist
  MISC_FEATURE (1): Xaa is 4-imidazoacetyl (CA)
XGQGTFTSDLSIQYDSEHQRDFIEWLKDTGPSSGAPPPSHG

SEQ ID NO: 20 - protein, 41 aa, Artificial Sequence
  Trigonal agonist
  MISC_FEATURE (1): Xaa is 4-imidazoacetyl (CA)
XGQGTFTSDLSIQYEEEAQQDFVEWLKDTGPSSGAPPPSHG

SEQ ID NO: 21 - protein, 39 aa, Artificial Sequence
  Trigonal agonist
  MISC_FEATURE (2): Xaa is aminoisobutyric acid (Aib)
  MISC_FEATURE (16)..(20): amino acids at positions 16 and 20 form a ring
YXQGTFTSDYSKYLDECRAKEFVQWLLDHHPSSGQPPPS

SEQ ID NO: 22 - protein, 39 aa, Artificial Sequence
  Trigonal agonist
  MISC_FEATURE (2): Xaa is aminoisobutyric acid (Aib)
  MISC_FEATURE (16)..(20): amino acids at positions 16 and 20 form a ring
YXQGTFTSDYSKCLDEKRAKEFVQWLLDHHPSSGQPPPS

SEQ ID NO: 23 - protein, 41 aa, Artificial Sequence
  Trigonal agonist
  MISC_FEATURE (2): Xaa is aminoisobutyric acid (Aib)
  MISC_FEATURE (16)..(20): amino acids at positions 16 and 20 form a ring
YXQGTFTSDYSKYLDECRAKEFVQWLLAQKGKKNDWKHNIT

SEQ ID NO: 24 - protein, 39 aa, Artificial Sequence
  Trigonal agonist
  MISC_FEATURE (2): Xaa is aminoisobutyric acid (Aib)
  MISC_FEATURE (16)..(20): amino acids at positions 16 and 20 form a ring
YXQGTFTSDYSKYLDECRAKEFVQWLKNGGPSSGAPPPS

SEQ ID NO: 25 - protein, 39 aa, Artificial Sequence
  Trigonal agonist
  MISC_FEATURE (2): Xaa is aminoisobutyric acid (Aib)
HXQGTFTSDCSKYLDERAAQDFVQWLLDGGPSSGAPPPS

SEQ ID NO: 26 - protein, 39 aa, Artificial Sequence
  Trigonal agonist
  MISC_FEATURE (2): Xaa is aminoisobutyric acid (Aib)
HXQGTFTSDCSKYLDSRAAQDFVQWLLDGGPSSGAPPPS

SEQ ID NO: 27 - protein, 40 aa, Artificial Sequence
  Trigonal agonist
  MISC_FEATURE (2): Xaa is aminoisobutyric acid (Aib)
HXQGTFTSDYSKYLDERACQDFVQWLLDQGGPSSGAPPPS

SEQ ID NO: 28 - protein, 41 aa, Artificial Sequence
  Trigonal agonist
  MISC_FEATURE (2): Xaa is aminoisobutyric acid (Aib)
HXQGTFTSDYSKYLDEKRAQEFVCWLLAQKGKKNDWKHNIT

SEQ ID NO: 29 - protein, 30 aa, Artificial Sequence
  Trigonal agonist
  MISC_FEATURE (2): Xaa is aminoisobutyric acid (Aib)
  MISC_FEATURE (16)..(20): amino acids at positions 16 and 20 form a ring
HXQGTFTSDYSKYLDEKAAKEFVQWLLNTC

SEQ ID NO: 30 - protein, 30 aa, Artificial Sequence
  Trigonal agonist
  MISC_FEATURE (2): Xaa is aminoisobutyric acid (Aib)
  MISC_FEATURE (16)..(20): amino acids at positions 16 and 20 form a ring
HXQGTFTSDYSKYLDEKAQKEFVQWLLDTC

SEQ ID NO: 31 - protein, 29 aa, Artificial Sequence
  Trigonal agonist
  MISC_FEATURE (2): Xaa is aminoisobutyric acid (Aib)
  MISC_FEATURE (16)..(20): amino acids at positions 16 and 20 form a ring
HXQGTFTSDYSKYLDEKACKEFVQWLLAQ

SEQ ID NO: 32 - protein, 39 aa, Artificial Sequence
  Trigonal agonist
  MISC_FEATURE (2): Xaa is aminoisobutyric acid (Aib)
  MISC_FEATURE (16)..(20): amino acids at positions 16 and 20 form a ring
HXQGTFTSDYSKYLDEKACKDFVQWLLDGGPSSGAPPPS

SEQ ID NO: 33 - protein, 31 aa, Artificial Sequence
  Trigonal agonist
  MISC_FEATURE (2): Xaa is aminoisobutyric acid (Aib)
  MISC_FEATURE (16)..(20): amino acids at positions 16 and 20 form a ring
HXQGTFTSDYSIAMDEIHQKDFVNWLLAQKC

SEQ ID NO: 34 - protein, 31 aa, Artificial Sequence
  Trigonal agonist
  MISC_FEATURE (2): Xaa is aminoisobutyric acid (Aib)
  MISC_FEATURE (16)..(20): amino acids at positions 16 and 20 form a ring
HXQGTFTSDYSKYLDEKRQKEFVNWLLAQKC

SEQ ID NO: 35 - protein, 31 aa, Artificial Sequence
  Trigonal agonist
  MISC_FEATURE (2): Xaa is aminoisobutyric acid (Aib)
  MISC_FEATURE (16)..(20): amino acids at positions 16 and 20 form a ring
HXQGTFTSDYSIAMDEIHQKDFVNWLLNTKC

SEQ ID NO: 36 - protein, 40 aa, Artificial Sequence
  Trigonal agonist
  MISC_FEATURE (2): Xaa is aminoisobutyric acid (Aib)
  MISC_FEATURE (16)..(20): amino acids at positions 16 and 20 form a ring
HXQGTFTSDYSKYLCEKRQKEFVQWLLNGGPSSGAPPPSG

SEQ ID NO: 37 - protein, 40 aa, Artificial Sequence
  Trigonal agonist
  MISC_FEATURE (2): Xaa is aminoisobutyric acid (Aib)
  MISC_FEATURE (16)..(20): amino acids at positions 16 and 20 form a ring
HXQGTFTSDYSKYLDECRQKEFVQWLLNGGPSSGAPPPSG

SEQ ID NO: 38 - protein, 40 aa, Artificial Sequence
  Trigonal agonist
  MISC_FEATURE (1): Xaa is 4-imidazoacetyl (CA)
  MISC_FEATURE (2): Xaa is aminoisobutyric acid (Aib)
XXQGTFTSDKSSYLDERAAQDFVQWLLDGGPSSGAPPPSS

SEQ ID NO: 39 - protein, 40 aa, Artificial Sequence
  Trigonal agonist
  MISC_FEATURE (2): Xaa is aminoisobutyric acid (Aib)
HXQGTFTSDYSKYLDGQHAQCFVAWLLAGGGPSSGAPPPS

SEQ ID NO: 40 - protein, 39 aa, Artificial Sequence
  Trigonal agonist
  MISC_FEATURE (2): Xaa is aminoisobutyric acid (Aib)
HXQGTFTSDKSKYLDERACQDFVQWLLDGGPSSGAPPPS

SEQ ID NO: 41 - protein, 39 aa, Artificial Sequence
  Trigonal agonist
  MISC_FEATURE (2): Xaa is aminoisobutyric acid (Aib)
HXQGTFTSDKSKYLDECAAQDFVQWLLDGGPSSGAPPPS

SEQ ID NO: 42 - protein, 40 aa, Artificial Sequence
  Trigonal agonist
  MISC_FEATURE (2): Xaa is aminoisobutyric acid (Aib)
  MISC_FEATURE (16)..(20): amino acids at positions 16 and 20 form a ring
YXQGTFTSDYSKYLDEKRAKEFVQWLLDHHPSSGQPPPSC

SEQ ID NO: 43 - protein, 39 aa, Artificial Sequence
  Trigonal agonist
  MISC_FEATURE (2): Xaa is aminoisobutyric acid (Aib)
  MISC_FEATURE (16)..(20): amino acids at positions 16 and 20 form a ring
YXQGTFTSDYSKYLDEKRAKEFVQWLLDHHCSSGQPPPS

SEQ ID NO: 44 - protein, 39 aa, Artificial Sequence
  Trigonal agonist
HGQGTFTSDCSKQLDGQAAQEFVAWLLAGGPSSGAPPPS

SEQ ID NO: 45 - protein, 39 aa, Artificial Sequence
  Trigonal agonist
HGQGTFTSDCSKYMDGQAAQDFVAWLLAGGPSSGAPPPS

SEQ ID NO: 46 - protein, 39 aa, Artificial Sequence
  Trigonal agonist
HGQGTFTSDCSKYLDEQHAQEFVAWLLAGGPSSGAPPPS

SEQ ID NO: 47 - protein, 39 aa, Artificial Sequence
  Trigonal agonist
HGQGTFTSDCSKYLDGQRAQEFVAWLLAGGPSSGAPPPS

SEQ ID NO: 48 - protein, 39 aa, Artificial Sequence
  Trigonal agonist
HGQGTFTSDCSKYLDGQRAQDFVNWLLAGGPSSGAPPPS

SEQ ID NO: 49 - protein, 30 aa, Artificial Sequence
  Trigonal agonist
  MISC_FEATURE (1): Xaa is 4-imidazoacetyl (CA)
  MISC_FEATURE (2): Xaa is aminoisobutyric acid (Aib)
  MISC_FEATURE (16)..(20): amino acids at positions 16 and 20 form a ring
XXQGTFTSDYSICMDEIHQKDFVNWLLNTK

SEQ ID NO: 50 - protein, 40 aa, Artificial Sequence
  Trigonal agonist
  MISC_FEATURE (2): Xaa is aminoisobutyric acid (Aib)
  MISC_FEATURE (16)..(20): amino acids at positions 16 and 20 form a ring
HXQGTFTSDYSKYLDEKRAKEFVQWLLDHHPSSGQPPPSC

SEQ ID NO: 51 - protein, 30 aa, Artificial Sequence
  Trigonal agonist
  MISC_FEATURE (2): Xaa is aminoisobutyric acid (Aib)
  MISC_FEATURE (16)..(20): amino acids at positions 16 and 20 form a ring
HXQGTFTSDYSKYLDEKRQKEFVQWLLNTC

SEQ ID NO: 52 - protein, 30 aa, Artificial Sequence
  Trigonal agonist
  MISC_FEATURE (2): Xaa is aminoisobutyric acid (Aib)
  MISC_FEATURE (16)..(20): amino acids at positions 16 and 20 form a ring
HXQGTFTSDYSKYLDEKRQKEFVQWLLDTC

SEQ ID NO: 53 - protein, 30 aa, Artificial Sequence
  Trigonal agonist
  MISC_FEATURE (2): Xaa is aminoisobutyric acid (Aib)
  MISC_FEATURE (16)..(20): amino acids at positions 16 and 20 form a ring
HXEGTFTSDYSIAMDEIHQKDFVNWLLAQC

SEQ ID NO: 54 - protein, 30 aa, Artificial Sequence
  Trigonal agonist
  MISC_FEATURE (2): Xaa is aminoisobutyric acid (Aib)
  MISC_FEATURE (16)..(20): amino acids at positions 16 and 20 form a ring
HXEGTFTSDYSIAMDEIHQKDFVDWLLAEC

SEQ ID NO: 55 - protein, 30 aa, Artificial Sequence
  Trigonal agonist
  MISC_FEATURE (2): Xaa is aminoisobutyric acid (Aib)
  MISC_FEATURE (16)..(20): amino acids at positions 16 and 20 form a ring
HXQGTFTSDYSIAMDEIHQKDFVNWLLAQC

SEQ ID NO: 56 - protein, 30 aa, Artificial Sequence
  Trigonal agonist
  MISC_FEATURE (2): Xaa is aminoisobutyric acid (Aib)
  MISC_FEATURE (16)..(20): amino acids at positions 16 and 20 form a ring
HXQGTFTSDYSKYLDEKRQKEFVNWLLAQC

SEQ ID NO: 57 - protein, 30 aa, Artificial Sequence
  Trigonal agonist
  MISC_FEATURE (2): Xaa is aminoisobutyric acid (Aib)
  MISC_FEATURE (16)..(20): amino acids at positions 16 and 20 form a ring
HXQGTFTSDYSIAMDEIHQKDFVNWLLNTC

SEQ ID NO: 58 - protein, 31 aa, Artificial Sequence
  Trigonal agonist
  MISC_FEATURE (2): Xaa is aminoisobutyric acid (Aib)
  MISC_FEATURE (16)..(20): amino acids at positions 16 and 20 form a ring
HXQGTFTSDYSKYLDEKRQKEFVQWLLNTKC

SEQ ID NO: 59 - protein, 30 aa, Artificial Sequence
  Trigonal agonist
  MISC_FEATURE (1): Xaa is 4-imidazoacetyl (CA)
  MISC_FEATURE (2): Xaa is aminoisobutyric acid (Aib)
  MISC_FEATURE (16)..(20): amino acids at positions 16 and 20 form a ring
XXQGTFTSDYSICMDEKHQKDFVNWLLNTK

SEQ ID NO: 60 - protein, 30 aa, Artificial Sequence
  Trigonal agonist
  MISC_FEATURE (1): Xaa is 4-imidazoacetyl (CA)
  MISC_FEATURE (2): Xaa is aminoisobutyric acid (Aib)
  MISC_FEATURE (16)..(20): amino acids at positions 16 and 20 form a ring
XXQGTFTSDYSIAMDEKHCKDFVNWLLNTK

SEQ ID NO: 61 - protein, 30 aa, Artificial Sequence
  Trigonal agonist
  MISC_FEATURE (1): Xaa is 4-imidazoacetyl (CA)
  MISC_FEATURE (2): Xaa is aminoisobutyric acid (Aib)
  MISC_FEATURE (16)..(20): amino acids at positions 16 and 20 form a ring
XXQGTFTSDYSIAMDEIACKDFVNWLLNTK

SEQ ID NO: 62 - protein, 39 aa, Artificial Sequence
  Trigonal agonist
  MISC_FEATURE (1): Xaa is 4-imidazoacetyl (CA)
  MISC_FEATURE (2): Xaa is aminoisobutyric acid (Aib)
XXQGTFTSDKSKYLDERAAQDFVQWLLDGGPSSGAPPPS

SEQ ID NO: 63 - protein, 39 aa, Artificial Sequence
  Trigonal agonist
  MISC_FEATURE (1): Xaa is 4-imidazoacetyl (CA)
  MISC_FEATURE (2): Xaa is aminoisobutyric acid (Aib)
XXQGTFTSDCSKYLDERAAQDFVQWLLDGGPSSGAPPPS

SEQ ID NO: 64 - protein, 39 aa, Artificial Sequence
  Trigonal agonist
  MISC_FEATURE (2): Xaa is aminoisobutyric acid (Aib)
  MISC_FEATURE (16)..(20): amino acids at positions 16 and 20 form a ring
YXQGTFTSDYSKYLDECAAKEFVQWLLDHHPSSGQPPPS

SEQ ID NO: 65 - protein, 39 aa, Artificial Sequence
  Trigonal agonist
  MISC_FEATURE (2): Xaa is aminoisobutyric acid (Aib)
  MISC_FEATURE (16)..(20): amino acids at positions 16 and 20 form a ring
HXQGTFTSDYSKCLDEKRAKEFVQWLLDHHPSSGQPPPS

SEQ ID NO: 66 - protein, 39 aa, Artificial Sequence
  Trigonal agonist
  MISC_FEATURE (2): Xaa is aminoisobutyric acid (Aib)
  MISC_FEATURE (16)..(20): amino acids at positions 16 and 20 form a ring
YXQGTFTSDYSKYLDECRAKDFVQWLLDHHPSSGQPPPS

SEQ ID NO: 67 - protein, 39 aa, Artificial Sequence
  Trigonal agonist
  MISC_FEATURE (2): Xaa is aminoisobutyric acid (Aib)
  MISC_FEATURE (16)..(20): amino acids at positions 16 and 20 form a ring
YXQGTFTSDYSKYLDECAAKDFVQWLLDHHPSSGQPPPS

SEQ ID NO: 68 - protein, 39 aa, Artificial Sequence
  Trigonal agonist
  MISC_FEATURE (2): Xaa is aminoisobutyric acid (Aib)
  MISC_FEATURE (16)..(20): amino acids at positions 16 and 20 form a ring
YXQGTFTSDYSKCLDEKAAKEFVQWLLDHHPSSGQPPPS

SEQ ID NO: 69 - protein, 39 aa, Artificial Sequence
  Trigonal agonist
  MISC_FEATURE (2): Xaa is aminoisobutyric acid (Aib)
  MISC_FEATURE (16)..(20): amino acids at positions 16 and 20 form a ring
YXQGTFTSDYSKCLDERAAKEFVQWLLDHHPSSGQPPPS

SEQ ID NO: 70 - protein, 39 aa, Artificial Sequence
  Trigonal agonist
  MISC_FEATURE (2): Xaa is aminoisobutyric acid (Aib)
  MISC_FEATURE (16)..(20): amino acids at positions 16 and 20 form a ring
YXQGTFTSDYSKCLDEKRAKDFVQWLLDHHPSSGQPPPS

SEQ ID NO: 71 - protein, 39 aa, Artificial Sequence
  Trigonal agonist
  MISC_FEATURE (2): Xaa is aminoisobutyric acid (Aib)
  MISC_FEATURE (16)..(20): amino acids at positions 16 and 20 form a ring
YXQGTFTSDYSKYLDERACKDFVQWLLDHHPSSGQPPPS

SEQ ID NO: 72 - protein, 39 aa, Artificial Sequence
  Trigonal agonist
  MISC_FEATURE (2): Xaa is aminoisobutyric acid (Aib)
  MISC_FEATURE (16)..(20): amino acids at positions 16 and 20 form a ring
YXQGTFTSDCSKYLDERAAKDFVQWLLDHHPSSGQPPPS

SEQ ID NO: 73 - protein, 39 aa, Artificial Sequence
  Trigonal agonist
  MISC_FEATURE (1): Xaa is 4-imidazoacetyl (CA)
  MISC_FEATURE (2): Xaa is aminoisobutyric acid (Aib)
  MISC_FEATURE (16)..(20): amino acids at positions 16 and 20 form a ring
XXQGTFTSDYSKYLDECRAKEFVQWLLDHHPSSGQPPPS

SEQ ID NO: 74 - protein, 39 aa, Artificial Sequence
  Trigonal agonist
  MISC_FEATURE (1): Xaa is 4-imidazoacetyl (CA)
  MISC_FEATURE (2): Xaa is aminoisobutyric acid (Aib)
  MISC_FEATURE (16)..(20): amino acids at positions 16 and 20 form a ring
XXQGTFTSDYSKCLDEKRAKEFVQWLLDHHPSSGQPPPS

SEQ ID NO: 75 - protein, 40 aa, Artificial Sequence
  Trigonal agonist
  MISC_FEATURE (2): Xaa is aminoisobutyric acid (Aib)
  MISC_FEATURE (16)..(20): amino acids at positions 16 and 20 form a ring
YXQGTFTSDYSKYLDEKAAKEFVQWLLDHHPSSGQPPPSC

SEQ ID NO: 76 - protein, 40 aa, Artificial Sequence
  Trigonal agonist
  MISC_FEATURE (2): Xaa is aminoisobutyric acid (Aib)
  MISC_FEATURE (16)..(20): amino acids at positions 16 and 20 form a ring
YXQGTFTSDYSKYLDEKRAKDFVQWLLDHHPSSGQPPPSC

SEQ ID NO: 77 - protein, 40 aa, Artificial Sequence
  Trigonal agonist
  MISC_FEATURE (2): Xaa is aminoisobutyric acid (Aib)
  MISC_FEATURE (16)..(20): amino acids at positions 16 and 20 form a ring
YXQGTFTSDYSKYLDEKAAKDFVQWLLDHHPSSGQPPPSC

SEQ ID NO: 78 - protein, 31 aa, Artificial Sequence
  Trigonal agonist
  MISC_FEATURE (2): Xaa is aminoisobutyric acid (Aib)
  MISC_FEATURE (16)..(20): amino acids at positions 16 and 20 form a ring
HXQGTFTSDYSKYLDEKRQKEFVQWLLDTKC

SEQ ID NO: 79 - protein, 31 aa, Artificial Sequence
  Trigonal agonist
  MISC_FEATURE (2): Xaa is aminoisobutyric acid (Aib)
  MISC_FEATURE (16)..(20): amino acids at positions 16 and 20 form a ring
HXEGTFTSDYSIAMDEIHQKDFVNWLLAQKC

SEQ ID NO: 80 - protein, 31 aa, Artificial Sequence
  Trigonal agonist
  MISC_FEATURE (2): Xaa is aminoisobutyric acid (Aib)
  MISC_FEATURE (16)..(20): amino acids at positions 16 and 20 form a ring
HXEGTFTSDYSIAMDEIHQKDFVDWLLAEKC

SEQ ID NO: 81 - protein, 30 aa, Artificial Sequence
  Trigonal agonist
  MISC_FEATURE (1): Xaa is 4-imidazoacetyl (CA)
  MISC_FEATURE (2): Xaa is aminoisobutyric acid (Aib)
  MISC_FEATURE (16)..(20): amino acids at positions 16 and 20 form a ring
XXQGTFTSDYSKYLDEKRQKEFVQWLLNTC

SEQ ID NO: 82 - protein, 30 aa, Artificial Sequence
  Trigonal agonist
  MISC_FEATURE (1): Xaa is 4-imidazoacetyl (CA)
  MISC_FEATURE (2): Xaa is aminoisobutyric acid (Aib)
  MISC_FEATURE (16)..(20): amino acids at positions 16 and 20 form a ring
XXQGTFTSDYSKYLDEKRQKEFVQWLLDTC

SEQ ID NO: 83 - protein, 30 aa, Artificial Sequence
  Trigonal agonist
  MISC_FEATURE (1): Xaa is 4-imidazoacetyl (CA)
  MISC_FEATURE (2): Xaa is aminoisobutyric acid (Aib)
  MISC_FEATURE (16)..(20): amino acids at positions 16 and 20 form a ring
XXEGTFTSDYSIAMDEIHQKDFVNWLLAQC

SEQ ID NO: 84 - protein, 30 aa, Artificial Sequence
  Trigonal agonist
  MISC_FEATURE (1): Xaa is 4-imidazoacetyl (CA)
  MISC_FEATURE (2): Xaa is aminoisobutyric acid (Aib)
  MISC_FEATURE (16)..(20): amino acids at positions 16 and 20 form a ring
XXEGTFTSDYSIAMDEIHQKDFVDWLLAEC

SEQ ID NO: 85 - protein, 30 aa, Artificial Sequence
  Trigonal agonist
  MISC_FEATURE (1): Xaa is 4-imidazoacetyl (CA)
  MISC_FEATURE (2): Xaa is aminoisobutyric acid (Aib)
  MISC_FEATURE (16)..(20): amino acids at positions 16 and 20 form a ring
XXQGTFTSDYSIAMDEIHQKDFVNWLLAQC

SEQ ID NO: 86 - protein, 30 aa, Artificial Sequence
  Trigonal agonist
  MISC_FEATURE (1): Xaa is 4-imidazoacetyl (CA)
  MISC_FEATURE (2): Xaa is aminoisobutyric acid (Aib)
  MISC_FEATURE (16)..(20): amino acids at positions 16 and 20 form a ring
XXQGTFTSDYSKYLDEKRQKEFVNWLLAQC

SEQ ID NO: 87 - protein, 30 aa, Artificial Sequence
  Trigonal agonist
  MISC_FEATURE (1): Xaa is 4-imidazoacetyl (CA)
  MISC_FEATURE (2): Xaa is aminoisobutyric acid (Aib)
  MISC_FEATURE (16)..(20): amino acids at positions 16 and 20 form a ring
XXQGTFTSDYSIAMDEIHQKDFVNWLLNTC

SEQ ID NO: 88 - protein, 31 aa, Artificial Sequence
  Trigonal agonist
  MISC_FEATURE (1): Xaa is 4-imidazoacetyl (CA)
  MISC_FEATURE (2): Xaa is aminoisobutyric acid (Aib)
  MISC_FEATURE (16)..(20): amino acids at positions 16 and 20 form a ring
XXQGTFTSDYSKYLDEKRQKEFVQWLLNTKC

SEQ ID NO: 89 - protein, 31 aa, Artificial Sequence
  Trigonal agonist
  MISC_FEATURE (1): Xaa is 4-imidazoacetyl (CA)
  MISC_FEATURE (2): Xaa is aminoisobutyric acid (Aib)
  MISC_FEATURE (16)..(20): amino acids at positions 16 and 20 form a ring
XXQGTFTSDYSKYLDEKRQKEFVQWLLDTKC

SEQ ID NO: 90 - protein, 31 aa, Artificial Sequence
  Trigonal agonist
  MISC_FEATURE (1): Xaa is 4-imidazoacetyl (CA)
  MISC_FEATURE (2): Xaa is aminoisobutyric acid (Aib)
  MISC_FEATURE (16)..(20): amino acids at positions 16 and 20 form a ring
XXEGTFTSDYSIAMDEIHQKDFVNWLLAQKC

SEQ ID NO: 91 - protein, 31 aa, Artificial Sequence
  Trigonal agonist
  MISC_FEATURE (1): Xaa is 4-imidazoacetyl (CA)
  MISC_FEATURE (2): Xaa is aminoisobutyric acid (Aib)
  MISC_FEATURE (16)..(20): amino acids at positions 16 and 20 form a ring
XXEGTFTSDYSIAMDEIHQKDFVDWLLAEKC

SEQ ID NO: 92 - protein, 31 aa, Artificial Sequence
  Trigonal agonist
  MISC_FEATURE (1): Xaa is 4-imidazoacetyl (CA)
  MISC_FEATURE (2): Xaa is aminoisobutyric acid (Aib)
  MISC_FEATURE (16)..(20): amino acids at positions 16 and 20 form a ring
XXQGTFTSDYSIAMDEIHQKDFVNWLLAQKC

SEQ ID NO: 93 - protein, 31 aa, Artificial Sequence
  Trigonal agonist
  MISC_FEATURE (1): Xaa is 4-imidazoacetyl (CA)
  MISC_FEATURE (2): Xaa is aminoisobutyric acid (Aib)
  MISC_FEATURE (16)..(20): amino acids at positions 16 and 20 form a ring
XXQGTFTSDYSKYLDEKRQKEFVNWLLAQKC

SEQ ID NO: 94 - protein, 31 aa, Artificial Sequence
  Trigonal agonist
  MISC_FEATURE (1): Xaa is 4-imidazoacetyl (CA)
  MISC_FEATURE (2): Xaa is aminoisobutyric acid (Aib)
  MISC_FEATURE (16)..(20): amino acids at positions 16 and 20 form a ring
XXQGTFTSDYSIAMDEIHQKDFVNWLLNTKC

SEQ ID NO: 95 - protein, 39 aa, Artificial Sequence
  Trigonal agonist
  MISC_FEATURE (2): Xaa is aminoisobutyric acid (Aib)
  MISC_FEATURE (16)..(20): amino acids at positions 16 and 20 form a ring
YXQGTFTSDYSKYLDEKRAKEFVQWLLCHHPSSGQPPPS

SEQ ID NO: 96 - protein, 39 aa, Artificial Sequence
  Trigonal agonist
  MISC_FEATURE (2): Xaa is aminoisobutyric acid (Aib)
  MISC_FEATURE (16)..(20): amino acids at positions 16 and 20 form a ring
YXQGTFTSDYSKYLDEKRAKEFVQWLLDHCPSSGQPPPS

SEQ ID NO: 97 - protein, 39 aa, Artificial Sequence
  Trigonal agonist
  MISC_FEATURE (2): Xaa is aminoisobutyric acid (Aib)
  MISC_FEATURE (16)..(20): amino acids at positions 16 and 20 form a ring
YXQGTFTSDYSKYLDEKRAKEFVQWLLDCHPSSGQPPPS

SEQ ID NO: 98 - protein, 40 aa, Artificial Sequence
  Trigonal agonist
  MISC_FEATURE (2): Xaa is aminoisobutyric acid (Aib)
  MISC_FEATURE (16)..(20): amino acids at positions 16 and 20 form a ring
YXQGTFTSDYSKALDEKAAKEFVNWLLDHHPSSGQPPPSC

SEQ ID NO: 99 - protein, 40 aa, Artificial Sequence
  Trigonal agonist
  MISC_FEATURE (2): Xaa is aminoisobutyric acid (Aib)
  MISC_FEATURE (16)..(20): amino acids at positions 16 and 20 form a ring
YXQGTFTSDYSKALDEKAAKDFVNWLLDHHPSSGQPPPSC

SEQ ID NO: 100 - protein, 40 aa, Artificial Sequence
  Trigonal agonist
  MISC_FEATURE (2): Xaa is aminoisobutyric acid (Aib)
  MISC_FEATURE (16)..(20): amino acids at positions 16 and 20 form a ring
YXQGTFTSDYSKALDEKAAKEFVQWLLDQHPSSGQPPPSC

SEQ ID NO: 101 - protein, 40 aa, Artificial Sequence
  Trigonal agonist
  MISC_FEATURE (2): Xaa is aminoisobutyric acid (Aib)
  MISC_FEATURE (16)..(20): amino acids at positions 16 and 20 form a ring
YXQGTFTSDYSKALDEKAAKEFVNWLLDQHPSSGQPPPSC

SEQ ID NO: 102 - protein, 40 aa, Artificial Sequence
  Trigonal agonist
  MISC_FEATURE (2): Xaa is aminoisobutyric acid (Aib)
  MISC_FEATURE (16)..(20): amino acids at positions 16 and 20 form a ring
YXQGTFTSDYSKALDEKAAKDFVNWLLDQHPSSGQPPPSC

SEQ ID NO: 103 - protein, 12 aa, HOMO SAPIENS
ESKYGPPCPSCP

SEQ ID NO: 104 - protein, 11 aa, Artificial Sequence
  Variant of hinge region
ESKYGPPPSCP

SEQ ID NO: 105 - protein, 11 aa, Artificial Sequence
  Variant of hinge region
ESKYGPPCPSP

SEQ ID NO: 106 - protein, 10 aa, Artificial Sequence
  Variant of hinge region
ESKYGPPCPS

SEQ ID NO: 107 - protein, 10 aa, Artificial Sequence
  Variant of hinge region
ESKYGPPCPP

SEQ ID NO: 108 - protein, 8 aa, Artificial Sequence
  Variant of hinge region
KYGPPCPS

SEQ ID NO: 109 - protein, 8 aa, Artificial Sequence
  Variant of hinge region
ESKYGPPC

SEQ ID NO: 110 - protein, 7 aa, Artificial Sequence
  Variant of hinge region
EKYGPPC

SEQ ID NO: 111 - protein, 6 aa, Artificial Sequence
  Variant of hinge region
ESPSCP

SEQ ID NO: 112 - protein, 5 aa, Artificial Sequence
  Variant of hinge region
EPSCP

SEQ ID NO: 113 - protein, 4 aa, Artificial Sequence
  Variant of hinge region
PSCP

SEQ ID NO: 114 - protein, 10 aa, Artificial Sequence
  Variant of hinge region
ESKYGPPSCP

SEQ ID NO: 115 - protein, 9 aa, Artificial Sequence
  Variant of hinge region
KYGPPPSCP

SEQ ID NO: 116 - protein, 9 aa, Artificial Sequence
  Variant of hinge region
ESKYGPSCP

SEQ ID NO: 117 - protein, 8 aa, Artificial Sequence
  Variant of hinge region
ESKYGPPC

SEQ ID NO: 118 - protein, 7 aa, Artificial Sequence
  Variant of hinge region
KYGPPCP

SEQ ID NO: 119 - protein, 7 aa, Artificial Sequence
  Variant of hinge region
ESKPSCP

SEQ ID NO: 120 - protein, 6 aa, Artificial Sequence
  Variant of hinge region
ESPSCP

SEQ ID NO: 121 - protein, 4 aa, Artificial Sequence
  Variant of hinge region
EPSC

SEQ ID NO: 122 - protein, 3 aa, Artificial Sequence
  Variant of hinge region
SCP

SEQ ID NO: 123 - protein, 221 aa, homo sapiens
PSCPAPEFLGGPSVFLFPPKPKDTLMISRTPEVTCVVVDVSQEDPEVQFNWYVDGVEVHNAKTKPREEQFNSTYRVVSVLTVLHQDWLNGKEYKCKVSNKGLPSSIEKTISKAKGQPREPQVYTLPPSQEEMTKNQVSLTCLVKGFYPSDIAVEWESNGQPENNYKTTPPVLDSDGSFFLYSRLTVDKSRWQEGNVFSCSVMHEALHNHYTQKSLSLSLGK

SEQ ID NO: 124 - protein, 442 aa, Homo sapiens
  MISC_FEATURE (1)..(442): Amino acids at position 1 to 442 form Human Immunoglobulin G4 Fc Fragment (homodimer)
  MISC_FEATURE (1)..(221): Amino acids at position 1 to 221 form one monomer
  MISC_FEATURE (222)..(442): Amino acids at position 222 to 442 form one monomer
  DISULFID (3)..(224): Amino acids at position 3 and position 224 form an inter-disulfide bond
  DISULFID (35)..(95): Amino acids at position 35 and position 95 form an intra-chain disulfide bond
  DISULFID (141)..(199): Amino acids at position 141 and position 199 form an intra-chain disulfide bond
  DISULFID (256)..(316): Amino acids at position 256 and position 316 form an intra-chain disulfide bond
  DISULFID (362)..(420): Amino acids at position 362 and position 420 form an intra-chain disulfide bond
PSCPAPEFLGGPSVFLFPPKPKDTLMISRTPEVTCVVVDVSQEDPEVQFNWYVDGVEVHNAKTKPREEQFNSTYRVVSVLTVLHQDWLNGKEYKCKVSNKGLPSSIEKTISKAKGQPREPQVYTLPPSQEEMTKNQVSLTCLVKGFYPSDIAVEWESNGQPENNYKTTPPVLDSDGSFFLYSRLTVDKSRWQEGNVFSCSVMHEALHNHYTQKSLSLSLGKPSCPAPEFLGGPSVFLFPPKPKDTLMISRTPEVTCVVVDVSQEDPEVQFNWYVDGVEVHNAKTKPREEQFNSTYRVVSVLTVLHQDWLNGKEYKCKVSNKGLPSSIEKTISKAKGQPREPQVYTLPPSQEEMTKNQVSLTCLVKGFYPSDIAVEWESNGQPENNYKTTPPVLDSDGSFFLYSRLTVDKSRWQEGNVFSCSVMHEALHNHYTQKSLSLSLGK